European Patent Application EP 4 530 352 A1, published April 2, 2025. Title: 바이러스 뉴클레오캡시드를 이용한 오량체형 독소 단백질 기반 목적 단백질 융합 오량체 제조 플랫폼. Applicant: 주식회사 백스다임. The sequence listing filed with the application follows.

SEQUENCE LISTING (17 sequences)

SEQ ID NO: 1 - protein, 54 aa, Human immunodeficiency virus 1
QRGNFRNQRKTVKCFNCGKEGHIAKNCRAPRKKGCWRCGREGHQMKDCTERQAN

SEQ ID NO: 2 - DNA, 162 bp, Human immunodeficiency virus 1
  source 1..162: mol_type = genomic DNA
cagcggggaaacttcaggaaccagagaaaaactgtgaagtgcttcaattgcggaaaggagggccacatcgctaagaactgccgcgcccccagaaagaaaggctgctggagatgcggcagagagggccaccagatgaaggactgcacagagagacaggcaaac

SEQ ID NO: 3 - DNA, 162 bp, synthetic construct
  source 1..162: mol_type = other DNA
cagcgtggtaacttccgtaaccagcgtaaaaccgttaaatgcttcaactgcggcaaagaaggccacatcgcgaaaaactgccgtgcgccgcgtaaaaaaggctgctggcgttgcggccgtgaaggccaccagatgaaagattgcaccgaacgtcaggcgaac

SEQ ID NO: 4 - protein, 103 aa, Escherichia coli
APQTITELCSEYRNTQIYTINDKILSYTESMAGKREMVIITFKSGETFQVEVPGSQHIDSQKKAIERMKDTLRITYLTETKIDKLCVWNNKTPNSIAAISMKN

SEQ ID NO: 5 - DNA, 309 bp, Escherichia coli
  source 1..309: mol_type = genomic DNA
gctccccagactattacagaactatgttcggaatatcgcaacacacaaatatatacgataaatgacaagatactatcatatacggaatcgatggcaggcaaaagagaaatggttatcattacatttaagagcggcgaaacatttcaggtcgaagtcccgggcagtcaacatatagactcccagaaaaaagccattgaaaggatgaaggacacattaagaatcacatatctgaccgagaccaaaattgataaattatgtgtatggaataataaaacccccaattcaattgcggcaatcagtatgaaaaac

SEQ ID NO: 6 - protein, 103 aa, Vibrio cholerae
TPQNITDLCAEYHNTQIHTLNDKIFSYTESLAGKREMAIITFKNGATFQVEVPGSQHIDSQKKAIERMKDTLRIAYLTEAKVEKLCVWNNKTPHAIAAISMAN

SEQ ID NO: 7 - DNA, 309 bp, Vibrio cholerae
  source 1..309: mol_type = genomic DNA
actccgcagaacattacggacctgtgtgcggagtatcataatacgcagattcacactttgaatgacaagattttttcatatacggagtcattagctggtaaacgtgaaatggcaattatcacttttaaaaatggtgcgacgttccaggtggaagttccgggcagtcagcatattgatagtcagaaaaaagccatcgaacgtatgaaggataccttgcgtattgcgtacttaaccgaggctaaagtcgagaaattatgtgtctggaataataagaccccacatgccattgctgcgatttcgatggccaat

SEQ ID NO: 8 - DNA, 480 bp, synthetic construct
  source 1..480: mol_type = other DNA
atgcagcggggaaacttcaggaaccagagaaaaactgtgaagtgcttcaattgcggaaaggagggccacatcgctaagaactgccgcgcccccagaaagaaaggctgctggagatgcggcagagagggccaccagatgaaggactgcacagagagacaggcaaacggatccgctccccagactattacagaactatgttcggaatatcgcaacacacaaatatatacgataaatgacaagatactatcatatacggaatcgatggcaggcaaaagagaaatggttatcattacatttaagagcggcgaaacatttcaggtcgaagtcccgggcagtcaacatatagactcccagaaaaaagccattgaaaggatgaaggacacattaagaatcacatatctgaccgagaccaaaattgataaattatgtgtatggaataataaaacccccaattcaattgcggcaatcagtatgaaaaac

SEQ ID NO: 9 - protein, 160 aa, synthetic construct
MQRGNFRNQRKTVKCFNCGKEGHIAKNCRAPRKKGCWRCGREGHQMKDCTERQANGSAPQTITELCSEYRNTQIYTINDKILSYTESMAGKREMVIITFKSGETFQVEVPGSQHIDSQKKAIERMKDTLRITYLTETKIDKLCVWNNKTPNSIAAISMKN

SEQ ID NO: 10 - DNA, 1446 bp, synthetic construct
  source 1..1446: mol_type = other DNA
cagcggggaaacttcaggaaccagagaaaaactgtgaagtgcttcaattgcggaaaggagggccacatcgctaagaactgccgcgcccccagaaagaaaggctgctggagatgcggcagagagggccaccagatgaaggactgcacagagagacaggcaaacgaaaacctgtattttcagggccatcaccatcaccatcacgatgatgatgatggtaccggatccgctccccagactattacagaactatgttcggaatatcgcaacacacaaatatatacgataaatgacaagatactatcatatacggaatcgatggcaggcaaaagagaaatggttatcattacatttaagagcggcgaaacatttcaggtcgaagtcccgggcagtcaacatatagactcccagaaaaaagccattgaaaggatgaaggacacattaagaatcacatatctgaccgagaccaaaattgataaattatgtgtatggaataataaaacccccaattcaattgcggcaatcagtatgaaaaacgatatcggcttaggtcagatgcttgaatccatgattgataacacagtgcgtgaaaccgtaggcgcagccacaagccgtgacgcgctgcctaacactgaagcgtctggtccgacgcactctaaagaaatcccggcgctgaccgcggttgaaaccggtgcgaccaacccgttagttccgtctgataccgttcagacccgtcacgttgttcagcaccgttctcgtagcgaatctagcattgaatctttcttcgcgcgtggtgcgtgcgtaacgatcatgaccgttgataacccagcgagcaccacaaacaaagataaattattcgctgtttggaaaatcacctacaaagataccgttcagctgcgtcgtaaactggaattcttcacctactctcgcttcgacatggaattgaccttcgttgttaccgcgaacttcaccgaaaccaacaacggtcacgcactgaaccaggtttaccagatcatgtacgttccgccgggcgcgccggttccggaaaaatgggatgattatacctggcagaccagcagcaacccgagcatcttctacacctacggtaccgcgccggcgcgtatcagcgttccgtacgtgggcatcagcaacgcgtatagccacttctatgacgggttcagcaaagttccgctgaaagatcagagcgcggcgctgggcgatagcctgtacggtgcggcgtccctgaacgatttcggtatcctggcggtgcgtgttgtgaacgatcacaacccgaccaaagtgacctctaaaatccgtgtttacctgaaaccgaaacacatccgtgtttggtgtccgcgtccgccgcgtgcggttgcgtactacggtccgggcgttgattacaaagatggtaccctgaccccgctgagcaccaaagatctgaccacctac

SEQ ID NO: 11 - protein, 482 aa, synthetic construct
QRGNFRNQRKTVKCFNCGKEGHIAKNCRAPRKKGCWRCGREGHQMKDCTERQANENLYFQGHHHHHHDDDDGTGSAPQTITELCSEYRNTQIYTINDKILSYTESMAGKREMVIITFKSGETFQVEVPGSQHIDSQKKAIERMKDTLRITYLTETKIDKLCVWNNKTPNSIAAISMKNDIGLGQMLESMIDNTVRETVGAATSRDALPNTEASGPTHSKEIPALTAVETGATNPLVPSDTVQTRHVVQHRSRSESSIESFFARGACVTIMTVDNPASTTNKDKLFAVWKITYKDTVQLRRKLEFFTYSRFDMELTFVVTANFTETNNGHALNQVYQIMYVPPGAPVPEKWDDYTWQTSSNPSIFYTYGTAPARISVPYVGISNAYSHFYDGFSKVPLKDQSAALGDSLYGAASLNDFGILAVRVVNDHNPTKVTSKIRVYLKPKHIRVWCPRPPRAVAYYGPGVDYKDGTLTPLSTKDLTTY

SEQ ID NO: 12 - DNA, 1446 bp, synthetic construct
  source 1..1446: mol_type = other DNA
cagcggggaaacttcaggaaccagagaaaaactgtgaagtgcttcaattgcggaaaggagggccacatcgctaagaactgccgcgcccccagaaagaaaggctgctggagatgcggcagagagggccaccagatgaaggactgcacagagagacaggcaaacgaaaacctgtattttcagggccatcaccatcaccatcacgatgatgatgatggtaccggatccactccgcagaacattacggacctgtgtgcggagtatcataatacgcagattcacactttgaatgacaagattttttcatatacggagtcattagctggtaaacgtgaaatggcaattatcacttttaaaaatggtgcgacgttccaggtggaagttccgggcagtcagcatattgatagtcagaaaaaagccatcgaacgtatgaaggataccttgcgtattgcgtacttaaccgaggctaaagtcgagaaattatgtgtctggaataataagaccccacatgccattgctgcgatttcgatggccaatgatatcggcttaggtcagatgcttgaatccatgattgataacacagtgcgtgaaaccgtaggcgcagccacaagccgtgacgcgctgcctaacactgaagcgtctggtccgacgcactctaaagaaatcccggcgctgaccgcggttgaaaccggtgcgaccaacccgttagttccgtctgataccgttcagacccgtcacgttgttcagcaccgttctcgtagcgaatctagcattgaatctttcttcgcgcgtggtgcgtgcgtaacgatcatgaccgttgataacccagcgagcaccacaaacaaagataaattattcgctgtttggaaaatcacctacaaagataccgttcagctgcgtcgtaaactggaattcttcacctactctcgcttcgacatggaattgaccttcgttgttaccgcgaacttcaccgaaaccaacaacggtcacgcactgaaccaggtttaccagatcatgtacgttccgccgggcgcgccggttccggaaaaatgggatgattatacctggcagaccagcagcaacccgagcatcttctacacctacggtaccgcgccggcgcgtatcagcgttccgtacgtgggcatcagcaacgcgtatagccacttctatgacgggttcagcaaagttccgctgaaagatcagagcgcggcgctgggcgatagcctgtacggtgcggcgtccctgaacgatttcggtatcctggcggtgcgtgttgtgaacgatcacaacccgaccaaagtgacctctaaaatccgtgtttacctgaaaccgaaacacatccgtgtttggtgtccgcgtccgccgcgtgcggttgcgtactacggtccgggcgttgattacaaagatggtaccctgaccccgctgagcaccaaagatctgaccacctac

SEQ ID NO: 13 - protein, 482 aa, synthetic construct
QRGNFRNQRKTVKCFNCGKEGHIAKNCRAPRKKGCWRCGREGHQMKDCTERQANENLYFQGHHHHHHDDDDGTGSTPQNITDLCAEYHNTQIHTLNDKIFSYTESLAGKREMAIITFKNGATFQVEVPGSQHIDSQKKAIERMKDTLRIAYLTEAKVEKLCVWNNKTPHAIAAISMANDIGLGQMLESMIDNTVRETVGAATSRDALPNTEASGPTHSKEIPALTAVETGATNPLVPSDTVQTRHVVQHRSRSESSIESFFARGACVTIMTVDNPASTTNKDKLFAVWKITYKDTVQLRRKLEFFTYSRFDMELTFVVTANFTETNNGHALNQVYQIMYVPPGAPVPEKWDDYTWQTSSNPSIFYTYGTAPARISVPYVGISNAYSHFYDGFSKVPLKDQSAALGDSLYGAASLNDFGILAVRVVNDHNPTKVTSKIRVYLKPKHIRVWCPRPPRAVAYYGPGVDYKDGTLTPLSTKDLTTY

SEQ ID NO: 14 - DNA, 1173 bp, synthetic construct
  source 1..1173: mol_type = other DNA
cagcggggaaacttcaggaaccagagaaaaactgtgaagtgcttcaattgcggaaaggagggccacatcgctaagaactgccgcgcccccagaaagaaaggctgctggagatgcggcagagagggccaccagatgaaggactgcacagagagacaggcaaacgaaaacctgtattttcagggccatcaccatcaccatcacgatgatgatgatggtaccggatccgctccccagactattacagaactatgttcggaatatcgcaacacacaaatatatacgataaatgacaagatactatcatatacggaatcgatggcaggcaaaagagaaatggttatcattacatttaagagcggcgaaacatttcaggtcgaagtcccgggcagtcaacatatagactcccagaaaaaagccattgaaaggatgaaggacacattaagaatcacatatctgaccgagaccaaaattgataaattatgtgtatggaataataaaacccccaattcaattgcggcaatcagtatgaaaaacgatatcaccactaccaccggtgaaagcgcagacccggtaactactaccgttgaaaactacgggggcgaaacccaaacggcgcgtcgtctgcatactgacgtagcgttcgtgctggaccgcttcgttaaactgacccaaccgaaatcaactcagacacttgatttaatgcagatcccttcccacaccctggtgggtgctctattgcgatctgccacctactacttcagcgatctggaagttgccctggtgcataccgggccggttacctgggttccgaacggcgctccgaaaaccgcactcaacaaccacaccaatccaacagcatatcagaaacagccgatcacccgtctggcgctgccttatactgccccgcatcgtgttctgagcacggtgtacaacggtaaaacgacctatggcgaagaatcgtctcgtcgtggtgacctggcggcgttggcacgtcgcgtgaataaccgcctgccgacctctttcaactacggtgcggtaaaagccgataccatcaccgaactgctgatccgtatgaaacgtgcggaaacctactgcccgcgcccgttgctggcactggataccacgcaggatcgccgtaaacaaaaaatcatcgcaccggaaaaacagatgatc

SEQ ID NO: 15 - protein, 391 aa, synthetic construct
QRGNFRNQRKTVKCFNCGKEGHIAKNCRAPRKKGCWRCGREGHQMKDCTERQANENLYFQGHHHHHHDDDDGTGSAPQTITELCSEYRNTQIYTINDKILSYTESMAGKREMVIITFKSGETFQVEVPGSQHIDSQKKAIERMKDTLRITYLTETKIDKLCVWNNKTPNSIAAISMKNDITTTTGESADPVTTTVENYGGETQTARRLHTDVAFVLDRFVKLTQPKSTQTLDLMQIPSHTLVGALLRSATYYFSDLEVALVHTGPVTWVPNGAPKTALNNHTNPTAYQKQPITRLALPYTAPHRVLSTVYNGKTTYGEESSRRGDLAALARRVNNRLPTSFNYGAVKADTITELLIRMKRAETYCPRPLLALDTTQDRRKQKIIAPEKQMI

SEQ ID NO: 16 - DNA, 1140 bp, synthetic construct
  source 1..1140: mol_type = other DNA
gctccccagactattacagaactatgttcggaatatcgcaacacacaaatatatacgataaatgacaagatactatcatatacggaatcgatggcaggcaaaagagaaatggttatcattacatttaagagcggcgaaacatttcaggtcgaagtcccgggcagtcaacatatagactcccagaaaaaagccattgaaaggatgaaggacacattaagaatcacatatctgaccgagaccaaaattgataaattatgtgtatggaataataaaacccccaattcaattgcggcaatcagtatgaaaaacggatccaccactaccaccggtgaaagcgcagacccggtaactactaccgttgaaaactacgggggcgaaacccaaacggcgcgtcgtctgcatactgacgtagcgttcgtgctggaccgcttcgttaaactgacccaaccgaaatcaactcagacacttgatttaatgcagatcccttcccacaccctggtgggtgctctattgcgatctgccacctactacttcagcgatctggaagttgccctggtgcataccgggccggttacctgggttccgaacggcgctccgaaaaccgcactcaacaaccacaccaatccaacagcatatcagaaacagccgatcacccgtctggcgctgccttatactgccccgcatcgtgttctgagcacggtgtacaacggtaaaacgacctatggcgaagaatcgtctcgtcgtggtgacctggcggcgttggcacgtcgcgtgaataaccgcctgccgacctctttcaactacggtgcggtaaaagccgataccatcaccgaactgctgatccgtatgaaacgtgcggaaacctactgcccgcgcccgttgctggcactggataccacgcaggatcgccgtaaacaaaaaatcatcgcaccggaaaaacagatgatcgatatccagcggggaaacttcaggaaccagagaaaaactgtgaagtgcttcaattgcggaaaggagggccacatcgctaagaactgccgcgcccccagaaagaaaggctgctggagatgcggcagagagggccaccagatgaaggactgcacagagagacaggcaaacaagcttcatcaccatcaccatcac

SEQ ID NO: 17 - protein, 380 aa, synthetic construct
APQTITELCSEYRNTQIYTINDKILSYTESMAGKREMVIITFKSGETFQVEVPGSQHIDSQKKAIERMKDTLRITYLTETKIDKLCVWNNKTPNSIAAISMKNGSTTTTGESADPVTTTVENYGGETQTARRLHTDVAFVLDRFVKLTQPKSTQTLDLMQIPSHTLVGALLRSATYYFSDLEVALVHTGPVTWVPNGAPKTALNNHTNPTAYQKQPITRLALPYTAPHRVLSTVYNGKTTYGEESSRRGDLAALARRVNNRLPTSFNYGAVKADTITELLIRMKRAETYCPRPLLALDTTQDRRKQKIIAPEKQMIDIQRGNFRNQRKTVKCFNCGKEGHIAKNCRAPRKKGCWRCGREGHQMKDCTERQANKLHHHHHH